European Patent Specification EP 3 894 861 B1, published July 10, 2024. Title: DETECTION OF BIOMARKERS FOR NON-SMALL CELL LUNG CANCER. Applicant: SENGENICS SDN BHD NATIONAL UNIVERSITY OF SINGAPORE. The sequence listing filed with the application follows.

SEQUENCE LISTING (38 sequences)

SEQ ID NO: 1 - DNA, 243 bp, Homo sapiens
atggaatcccccaagaagaagaaccagcagctgaaggtcggaatcctgcacctgggttcccgtcagaagaagatccgtatccagctgcgttcccagtgcgctacctggaaggtcatctgcaagtcctgcatctcccagacccccggtatcaacctggacctgggctccggtgtcaaggtcaagatcatccccaaggaagaacactgcaagatgcccgaggctggcgaggaacagccccaggtg

SEQ ID NO: 2 - DNA, 1200 bp, Homo sapiens
atggggactcctgcttctggaaggaaaagaacacctgtgaaagaccgattttctgcagaagatgaagctttgagtaacattgccagagaggcagaggcaaggctggcagcaaaacgggctgcccgggcagaagcaagagatatacgcatgagagaactggaacgacaacaaaaagagttggatgaaaaatctgacaaacagtatgctgaaaattatacaagaccttcatctcgaaattctgcctcagcaacaacccctctaagtggaaactcatccagacgaggaagtggggacaccagcagcttaatagatccagacacttcattaagtgaattgcgggaatctttgtctgaagtggaagaaaaatacaagaaagccatggtttccaatgcacagttagacaatgagaagaacaatttgatctaccaagtagacacactcaaggatgttattgaagagcaggaggaacagatggcagaattttatagagaaaatgaagaaaaatcaaaggagttagaaaggcagaaacatatgtgtagtgtgctgcagcataagatggaagaacttaaagaaggcctgcggcaaagagatgagcttattgagaaacatggcttagttataatccccgatggcactcccaatggtgatgtcagtcatgaaccagtggctggagccatcactgttgtgtctcaggaagctgctcaggtcttggagtcagcaggagaagggccattagatgtaaggctacgaaaacttgctggagagaaggaagaactactgtcacagattagaaaactgaagcttcagttagaggaggaacgacagaaatgctccaggaatgatggcacagtgggtgacctggcaggactgcagaatggctcagacttgcagttcatcgaaatgcagagagatgccaatagacaaattagcgaatacaaatttaagctttcaaaagcagaacaggatataactaccttggagcaaagtattagccggcttgagggacaggttctgagatataaaactgctgctgagaatgctgagaaagttgaagatgaattgaaagcagaaaaacggaagctacaacgagagttacgaacagcactggacaagattgaggagatggagatgaccaacagccacctggccaagcggctggagaagatgaaggccaataggacagcacttctggcccagcag

SEQ ID NO: 3 - DNA, 348 bp, Homo sapiens
atgtcctggcgtggtcgttccacctaccgtccccgtcctcgtcgttacgtcgagccccccgagatgatcggtcccatgcgtcccgagcagttctccgacgaggtcgagcccgctacccccgaggaaggcgagcctgctactcagcgtcaggaccccgctgctgctcaagagggcgaggacgagggcgcttccgctggccagggtcctaagcccgaggctcactcccaagagcagggtcacccccagaccggttgcgagtgcgaggacggtcccgacggtcaagagatggacccccccaaccctgaggaagtcaagacccccgaagagggcgaaaagcagtcccagtgc

SEQ ID NO: 4 - DNA, 1893 bp, Homo sapiens
atgtcccactgggctcccgagtggaagcgtgctgaggctaacccccgtgacctgggcgcttcttgggacgtgcgcggttcccgtggtagcggttggagcggtcccttcggtcaccaaggtccccgtgctgctggttcccgcgagccccccctgtgcttcaagatcaagaacaacatggtcggagtggtcatcggttactccggttccaagatcaaggacctgcagcactccaccaacaccaagatccagatcatcaacggcgagtccgaggctaaggtccgcatcttcggcaaccgcgagatgaaggctaaggccaaggctgctatcgagactctgatccgcaagcaagagtcctacaactccgagtcctccgtggacaacgctgcttcccagacccccatcggtcgtaacctgggtcgtaacgacatcgtgggcgaggctgagcccctgtccaactgggaccgtatccgcgctgctgtggtcgagtgcgagaagcgcaagtgggctgacctgccccccgtgaagaagaacttctacatcgagtccaaggctacctcctgcatgtccgagatgcaagtgatcaactggcgcaaggaaaacttcaacatcacttgcgacgacctgaagtccggcgagaagcgtctgatccccaagcctacctgccgtttcaaggacgctttccagcagtaccccgacctgctgaagtccatcatccgtgtgggtatcgtgaagcccacccccatccagtcccaggcttggccaatcatcctgcagggtatcgacctgatcgtggtggctcagaccggcaccggcaagaccctgtcctacctgatgcccggtttcatccacctggactcccagcccatctcccgcgagcagcgtaacggtcccggcatgctggtgctgacccctacccgtgaactggctctgcacgtcgaggctgagtgctccaagtactcctacaagggcctgaagtctatctgcatctacggtggtcgtaaccgtaacggccagatcgaggacatctccaagggtgtcgacatcatcattgctacccccggtcgtctgaacgacctgcagatgaacaactccgtgaacctgcgttccatcacctacctggtcatcgacgaggctgacaagatgctggacatggagttcgagccccagatccgcaagatcctgctggacgtgcgtcccgaccgtcagaccgtgatgacctccgctacctggcccgacaccgtgcgtcagctggctctgtcttacctgaaggaccccatgatcgtgtacgtgggcaacctgaacctggtggctgtgaacaccgtgaagcagaacatcatcgtgaccaccgagaaggaaaagagggctctgacccaagagttcgtcgagaacatgtcccccaacgacaaggtcatcatgttcgtgtcccagaagcacattgctgacgacctgtcctccgatttcaacatccaaggcatctccgctgagtccctgcacggcaactccgagcagtccgaccaagagcgtgctgtcgaggacttcaagtccggcaacatcaagatcctcatcaccaccgacatcgtgtcccgtggcctggacctgaacgacgtgacccacgtgtacaactacgacttcccccgtaacatcgacgtgtacgtgcaccgtgtgggttacatcggtcgcaccggaaagaccggaacctccgtgaccctgatcacccagcgcgactccaagatggctggcgagctgatcaagatcttggaccgtgctaaccagtccgtgcccgaggacctggtggtcatggctgagcagtacaagctgaaccagcagaagcgtcaccgcgagactcgttcccgcaagcccggacagcgtcgcaaggagttctacttcctgtcc

SEQ ID NO: 5 - DNA, 1944 bp, Homo sapiens
atgtcccaccacggtggtgctcccaaggcttccacctgggtggtggcttcccgtcgttcctccaccgtgtcccgtgctcccgagcgtcgtcccgctgaggaactgaaccgtaccggtcccgagggctactccgtgggtcgtggtggtcgttggcgtggcacctctcgtccccctgaggctgtggctgctggtcacgaggaactgcccctgtgcttcgctctgaagtcccacttcgtgggtgctgtgatcggtcgcggtggttccaagatcaagaacatccagtccaccaccaacaccaccatccagatcatccaagagcagcccgagtccctggtcaagatcttcggttccaaggctatgcagaccaaggctaaggctgtgatcgacaacttcgtgaagaagctggaagagaactacaactccgagtgcggtatcgacaccgctttccagccctccgtgggcaaggacggttccaccgacaacaacgtggtggctggcgaccgtcccctgatcgactgggaccagatccgtgaagagggcctgaagtggcaaaagaccaagtgggctgacctgccccccatcaagaagaacttctacaaggaatccaccgctacctccgctatgtccaaggtcgaggctgactcctggcgcaaggaaaacttcaacatcacctgggacgacctgaaggacggcgagaagcgtcccatccccaaccctacctgcaccttcgacgacgctttccagtgctaccccgaagtgatggaaaacatcaagaaggctggtttccagaagcccacccccatccagtcccaggcttggcccatcgtgctgcagggtatcgacctgatcggtgtcgctcagaccggcaccggcaagaccctgtgctacctgatgcccggtttcatccacctggtgctgcagccctccctgaagggccagcgtaaccgtcccggcatgctggtgctgacccctacccgcgaactggctctgcaggtcgagggcgagtgctgcaagtactcctacaagggcctgcgttccgtgtgcgtgtacggtggtggcaaccgtgacgagcagatcgaggaactcaagaagggtgtcgacatcatcatcgctacccccggtcgtctgaacgacctgcagatgtccaacttcgtcaacctgaagaacatcacctacctggtcctggacgaggctgacaagatgctggacatgggtttcgagccccagatcatgaagatcctgctggacgtgcgtcccgaccgtcagaccgtgatgacctccgctacctggccccactccgtgcaccgtctggctcagtcctacctgaaggaacccatgatcgtgtacgtgggcaccctggacctggtggctgtgtcctccgtgaagcagaacatcatcgtgaccaccgaggaagagaagtggtcccacatgcagactttcttgcagtccatgtcctctaccgacaaggtcatcgtgttcgtgtcccgcaaggctgtcgctgaccacctgtcctccgacctgatcctgggcaacatctccgtcgagtccctgcacggcgaccgcgagcagcgtgaccgcgagaaggctctcgagaacttcaagaccggcaaggtccgcatcctgatcgctaccgacctggcttcccgcggactggacgtgcacgacgtgacccacgtgtacaacttcgacttcccccgtaacatcgaggaatacgtgcaccgtatcggtcgtaccggtcgtgctggtcgcaccggtgtctccatcaccaccctgacccgtaacgactggcgtgtggcttccgagctgatcaacatcctcgagcgtgctaaccagtccatccccgaggaactggtgtctatggctgagcgtttcaaggctcaccagcaaaagcgcgagatggaacgcaagatggaacgtccccagggtcgtcccaagaagttccac

SEQ ID NO: 6 - DNA, 351 bp, Homo sapiens
atgtcctggcgtggtcgttccacctactactggccccgtccccgtcgttacgtgcagccccccgagatgatcggtcccatgcgtcccgagcagttctccgacgaggtcgagcccgctacccccgaggaaggcgagcctgctactcagcgtcaggaccccgctgctgctcaagagggcgaggacgagggcgcttccgctggccagggtcctaagcccgaggctgactcccaagagcagggtcacccccagaccggttgcgagtgcgaggacggtcccgacggtcaagagatggacccccccaaccctgaggaagtcaagacccccgaagagggcgaaggccagtcccagtgc

SEQ ID NO: 7 - DNA, 1107 bp, Homo sapiens
atgccccgtgctcccaagcgtcagcgttgcatgcccgaagaggacctgcagtcccagtccgagactcagggcctcgagggtgctcaggctcccctggctgtggaagaggacgcttccagctctacctctacctcctccagcttccccagcagcttcccatcctccagctcctctagctcctcctcctgctaccccctgatcccctccacccccgaggaagtgtccgctgacgacgagactcccaaccccccccagtccgctcagatcgcttgctcctccccctccgtggtggcttccctgcctctggaccagtccgacgagggttccagctcccagaaggaagagtcccccagcaccctgcaggtcctgcccgactccgagtccctgccccgttccgagatcgacgagaaggttacagacctggtgcagttcctgctgttcaagtaccagatgaaggaacccatcaccaaggctgagatcctcgagtccgtgatcaagaactacgaggaccacttccccctgctgttctccgaggcttccgagtgcatgctgctggtgttcggtatcgacgtgaaggaagtggaccctaccggtcactccttcgtgctggtcacctccctgggcctgacctacgacggcatgctgtccgacgtgcagtccatgcccaagaccggtatcctgatcctcatcctgtccatcatcttcatcgagggctactgcactcctgaggaagtgatctgggaggctctgaacatgatgggcctgtacgacggaatggaacacctgatctacggcgagccccgcaagctgctgacccaggactgggtgcaagagaactacctcgagtaccgtcaggtgcccggttccgaccccgctcgttacgagttcctgtggggtccccgtgctcacgctgagatccgcaagatgtccctgctgaagttcctggctaaggtcaacggctccgacccccgttccttcccactgtggtacgaggaagctctgaaggacgaggaagagagggctcaggaccgtatcgctaccaccgacgacaccaccgctatggcttccgcttcctctagcgctaccggttccttcagctaccccgag

SEQ ID NO: 8 - DNA, 378 bp, Homo sapiens
atgtctgtcatggacctcgccaatacttgctccagctttcagtcggacctggatttctgttcagattgcggctcggtcctgcctctgcccggggctcaggatacggtcacctgtattcgctgtggcttcaacatcaacgttcgggactttgaggggaaggttgtgaagacttcggttgtgttccaccaactggggacagccatgcctatgtcggtggaggaagggcctgagtgccagggacctgtggttgacaggcgctgccctcgatgtggtcatgaaggaatggcataccacaccagacagatgcgttcagccgatgaagggcaaactgtcttctacacctgtaccaactgcaagttccaggagaaggaagactct

SEQ ID NO: 9 - DNA, 1344 bp, Homo sapiens
atgctgtggctagcccttggcccctttcctgccatggagaaccaggtgctggtaattcgcatcaagatcccaaatagtggcgcggtggactggacagtgcactccgggccgcagttactcttcagggatgtgctggatgtgataggccaggttctgcctgaagcaacaactacagcatttgaatatgaagatgaagatggtgatcgaattacagtgagaagtgatgaggaaatgaaggcaatgctgtcatattattattccacagtaatggaacagcaagtaaatggacagttaatagagcctctgcagatatttccaagagcctgcaagcctcctggggaacggaacatacatggcctgaaggtgaatactcgggccggaccctctcaacacagcagcccagcagtctcagattcacttccaagcaatagcttaaagaagtcttctgctgaactgaaaaaaatactagccaatggccagatgaatgaacaagacatacgatatcgggacactcttggtcatggcaacggaggcacagtctacaaagcatatcatgtcccgagtgggaaaatattagctgtaaaggtcatactactagatattacactggaacttcagaagcaaattatgtctgaattggaaattctttataagtgcgattcatcatatatcattggattttatggagcattttttgtagaaaacaggatttcaatatgtacagaattcatggatgggggatctttggatgtatataggaaaatgccagaacatgtccttggaagaattgcagtagcagttgttaaaggccttacttatttgtggagtttaaagattttacatagagacgtgaagccctccaatatgctagtaaacacaagaggacaggttaagctgtgtgattttggagttagcactcagctggtgaattctatagccaagacgtatgttggaacaaatgcttatatggcgcctgaaaggatttcaggggagcagtatggaattcattctgatgtctggagcttaggaatctcttttatggagcttgctcttgggaggtttccatatcctcagattcagaaaaaccagggatctttaatgcctctccagcttctgcagtgcattgttgatgaggattcgcccgtccttccagttggagagttctcggagccatttgtacatttcatcactcagtgtatgcgaaaacagccaaaagaaaggccagcacctgaagaattgatgggccacccgttcatcgtgcagttcaatgatggaaatgccgccgtggtgtccatgtgggtgtgccgggcgctggaggagaggcggagccagcaggggcccccg

SEQ ID NO: 10 - DNA, 951 bp, Homo sapiens
atgtcttctgagcagaagagtcagcactgcaagcctgaggaaggcgttgaggcccaagaagaggccctgggcctggtgggtgcacaggctcctactactgaggagcaggaggctgctgtctcctcctcctctcctctggtccctggcaccctggaggaagtgcctgctgctgagtcagcaggtcctccccagagtcctcagggagcctctgccttacccactaccatcagcttcacttgctggaggcaacccaatgagggttccagcagccaagaagaggaggggccaagcacctcgcctgacgcagagtccttgttccgagaagcactcagtaacaaggtggatgagttggctcattttctgctccgcaagtatcgagccaaggagctggtcacaaaggcagaaatgctggagagagtcatcaaaaattacaagcgctgctttcctgtgatcttcggcaaagcctccgagtccctgaagatgatctttggcattgacgtgaaggaagtggaccccaccagcaacacctacacccttgtcacctgcctgggcctttcctatgatggcctgctgggtaataatcagatctttcccaagacaggccttctgataatcgtcctgggcacaattgcaatggagggcgacagcgcctctgaggaggaaatctgggaggagctgggtgtgatgggggtgtatgatgggagggagcacactgtctatggggagcccaggaaactgctcacccaagattgggtgcaggaaaactacctggagtaccggcaggtacccggcagtaatcctgcgcgctatgagttcctgtggggtccaagggctctggctgaaaccagctatgtgaaagtcctggagcatgtggtcagggtcaatgcaagagttcgcattgcctacccatccctgcgtgaagcagctttgttagaggaggaagagggagtc

SEQ ID NO: 11 - DNA, 2136 bp, Homo sapiens
atgtctcagtggtacgaacttcagcagcttgactcaaaattcctggagcaggttcaccagctttatgatgacagttttcccatggaaatcagacagtacctggcacagtggttagaaaagcaagactgggagcacgctgccaatgatgtttcatttgccaccatccgttttcatgacctcctgtcacagctggatgatcaatatagtcgcttttctttggagaataacttcttgctacagcataacataaggaaaagcaagcgtaatcttcaggataattttcaggaagacccaatccagatgtctatgatcatttacagctgtctgaaggaagaaaggaaaattctggaaaacgcccagagatttaatcaggctcagtcggggaatattcagagcacagtgatgttagacaaacagaaagagcttgacagtaaagtcagaaatgtgaaggacaaggttatgtgtatagagcatgaaatcaagagcctggaagatttacaagatgaatatgacttcaaatgcaaaaccttgcagaacagagaacacgagaccaatggtgtggcaaagagtgatcagaaacaagaacagctgttactcaagaagatgtatttaatgcttgacaataagagaaaggaagtagttcacaaaataatagagttgctgaatgtcactgaacttacccagaatgccctgattaatgatgaactagtggagtggaagcggagacagcagagcgcctgtattggggggccgcccaatgcttgcttggatcagctgcagaactggttcactatagttgcggagagtctgcagcaagttcggcagcagcttaaaaagttggaggaattggaacagaaatacacctacgaacatgaccctatcacaaaaaacaaacaagtgttatgggaccgcaccttcagtcttttccagcagctcattcagagctcgtttgtggtggaaagacagccctgcatgccaacgcaccctcagaggccgctggtcttgaagacaggggtccagttcactgtgaagttgagactgttggtgaaattgcaagagctgaattataatttgaaagtcaaagtcttatttgataaagatgtgaatgagagaaatacagtaaaaggatttaggaagttcaacattttgggcacgcacacaaaagtgatgaacatggaggagtccaccaatggcagtctggcggctgaatttcggcacctgcaattgaaagaacagaaaaatgctggcaccagaacgaatgagggtcctctcatcgttactgaagagcttcactcccttagttttgaaacccaattgtgccagcctggtttggtaattgacctcgagacgacctctctgcccgttgtggtgatctccaacgtcagccagctcccgagcggttgggcctccatcctttggtacaacatgctggtggcggaacccaggaatctgtccttcttcctgactccaccatgtgcacgatgggctcagctttcagaagtgctgagttggcagttttcttctgtcaccaaaagaggtctcaatgtggaccagctgaacatgttgggagagaagcttcttggtcctaacgccagccccgatggtctcattccgtggacgaggttttgtaaggaaaatataaatgataaaaattttcccttctggctttggattgaaagcatcctagaactcattaaaaaacacctgctccctctctggaatgatgggtgcatcatgggcttcatcagcaaggagcgagagcgtgccctgttgaaggaccagcagccggggaccttcctgctgcggttcagtgagagctcccgggaaggggccatcacattcacatgggtggagcggtcccagaacggaggcgaacctgacttccatgcggttgaaccctacacgaagaaagaactttctgctgttactttccctgacatcattcgcaattacaaagtcatggctgctgagaatattcctgagaatcccctgaagtatctgtatccaaatattgacaaagaccatgcctttggaaagtattactccaggccaaaggaagcaccagagccaatggaacttgatggccctaaaggaactggatatatcaagactgagttgatttctgtgtctgaagtg

SEQ ID NO: 12 - DNA, 864 bp, Homo sapiens
atgtccgctaccggcgaccgtcaccctacccagggcgaccaagaggctcccgtgtcccaagagggtgctcaggctgaggctgctggtgctggcaaccaggaaggtggcgactccggtcccgactcctccgacgtggtgcctgctgctgaggtcgtgggtgtcgctggtcctgtcgagggcctgggagaggaagagggcgagcaggctgctggcctggctgctgtgcctcgtggtggttccgctgaagaggactccgacatcggtcccgctaccgaggaagaggaagaagaagagggcaacgaggctgctaacttcgacctggctgtggtggctcgtcgttaccccgcttccggtatccacttcgtgctgctggacatggtgcactccctgctgcaccgtctgtcccacaacgaccacatcctgatcgagaaccgtcagctgtcccgtctgatggtcggaccccacgctgctgctcgtaacctgtggggcaacctgccccccctgctgctgcctcaacgtctgggagctggtgctgctgctagggctggcgagggactgggcctgatccaagaggctgcttccgtgcccgagcccgctgtgcctgctgacttggctgagatggcccgcgagcctgctgaggaagctgctgaagagaagctgtccgaggaagccaccgaggaacccgacgctgaggaaccagctactgaggaacccaccgctcaagaggctaccgctcctgaggaagtgaccaagtcccagcccgagaagtgggacgaggaagctcaggacgctgctggcgaggaagagaaggaacaagaaaaggaaaaggacgccgagaacaaggtcaagaactccaagggcacc

SEQ ID NO: 13 - DNA, 1737 bp, Homo sapiens
atgaacaagctgtacatcggcaacctgtccgagaacgctgctccctccgacctcgagtccatcttcaaggacgctaagatccccgtgtccggacccttcctggtcaagaccggttacgctttcgtggactgccccgacgagtcctgggctctgaaggctatcgaggctctgtccggcaagatcgagctgcacggcaagcccatcgaggtcgagcactccgtgcccaagcgtcagcgtatccgcaagctgcagatccgtaacatccccccacacctccagtgggaggtgctggactccctgctggtgcagtacggtgtcgtcgagtcctgcgagcaagtgaacaccgactccgagactgctgtggtcaacgtgacctactcctccaaggaccaggctcgtcaggctctggacaagctgaacggtttccagctcgagaacttcaccctgaaggtggcctacatccccgacgagatggctgctcagcagaaccccctgcagcagccccgtggtcgtcgtggactgggacagcgtggtagctcccgtcagggttcccccggttccgtgtccaagcagaagccctgcgacctgcccctgcgtctgctggtgcctacccagttcgtgggtgctatcatcggcaaggaaggtgctaccatccgcaacatcaccaagcagacccagtccaagatcgacgtccaccgcaaggaaaacgctggcgctgctgagaagtccatcaccatcctgtccacccccgagggcacctccgctgcttgcaagtccatcctcgagatcatgcacaaggaagcccaggacatcaagttcaccgaggaaatccccctgaagatcctggctcacaacaacttcgtgggtcgtctgatcggaaaggaaggccgtaacctgaagaagatcgagcaggacaccgacaccaagatcaccatctccccactgcaagagctgaccctgtacaaccccgagcgtaccatcaccgtgaagggcaacgtggaaacctgcgctaaggctgaagaggaaatcatgaagaagatccgcgagtcctacgagaacgatatcgcttccatgaacctgcaggctcacctgatccccggcctgaacctgaacgctctgggcctgttcccccctacctccggcatgcctcctcccacctctggtcccccctccgctatgacccccccatacccccagttcgagcagtccgagactgagactgtgcacctgttcatccccgctctgtccgtcggtgccatcatcggaaagcagggccagcacatcaagcagctgtcccgtttcgctggtgcttccatcaagatcgctcccgctgaggctcccgacgctaaggtccgcatggtcatcatcaccggtccccccgaggctcagttcaaggctcagggtcgtatctacggcaagatcaaggaagagaacttcgtcagccccaaggaagaagtgaagctcgaggctcacatccgtgtgccatccttcgctgctggtcgtgttatcggcaagggtggcaagaccgtgaacgagctgcagaacctgtcctccgctgaggtggtggtgccccgtgaccagacccctgacgagaacgaccaggtggtggtcaagatcaccggtcacttctacgcttgccaggtggcccagcgcaagatccaagagatcctgacccaagtgaagcagcaccagcagcagaaggctctgcagtccggtccccctcagtcccgtcgcaag

SEQ ID NO: 14 - DNA, 630 bp, Homo sapiens
atgcaggccgaaggccggggcacagggggttcgacgggcgatgctgatggcccaggaggccctggcattcctgatggcccagggggcaatgctggcggcccaggagaggcgggtgccacgggcggcagaggtccccggggcgcaggggcagcaagggcctcggggccgagaggaggcgccccgcggggtccgcatggcggtgccgcttctgcgcaggatggaaggtgcccctgcggggccaggaggccggacagccgcctgcttgagttgcacatcacgatgcctttctcgtcgcccatggaagcggagctggtccgcaggatcctgtcccgggatgccgcaccgctcccccgaccaggggcggttctgaaggacttcaccgtgtccggcaacctactgtttatgtcagttcgggaccaggacagggaaggcgctgggcggatgagggtggtgggttgggggctgggatccgcctccccggaggggcagaaagctagagatctcagaacacccaaacacaaggtctcagaacagagacctggtacaccaggcccgccgccacccgagggagcccagggagatgggtgcagaggtgtcgcctttaatgtgatgttctctgcccctcacatt

SEQ ID NO: 15 - DNA, 1227 bp, Homo sapiens
atgcaggtcaccctgaagaccctccagcagcagaccttcaagatagacattgaccccgaggagacggtgaaagcactgaaagagaagattgaatctgaaaaggggaaagatgcctttccagtagcaggtcaaaaattaatttatgcaggcaaaatcctcaatgatgatactgctctcaaagaatataaaattgatgagaaaaactttgtggtggttatggtgaccaaacccaaagcagtgtccacaccagcaccagctacaactcagcagtcagctcctgccagcactacagcagttacttcctccaccaccacaactgtggctcaggctccaacccctgtccctgccttggcccccacttccacacctgcatccatcactccagcatcagcgacagcatcttctgaacctgcacctgctagtgcagctaaacaagagaagcctgcagaaaagccagcagagacaccagtggctactagcccaacagcaactgacagtacatcgggtgattcttctcggtcaaacctttttgaagatgcaacgagtgcacttgtgacgggtcagtcttacgagaatatggtaactgagatcatgtcaatgggctatgaacgagagcaagtaattgcagccctgagagccagtttcaacaaccctgacagagcagtggagtatcttttaatgggaatccctggagatagagaaagtcaggctgtggttgacccccctcaagcagctagtactggggttcctcagtcttcagcagtggctgcagctgcagcaactacgacagcaacaactacaacaacaagttctggaggacatccccttgaatttttacggaatcagcctcagtttcaacagatgagacaaattattcagcagaatccttccttgcttccagcgttactacagcagataggtcgagagaatcctcaattacttcagcaaattagccaacaccaggagcattttattcagatgttaaatgaaccagttcaagaagctggtggtcaaggaggaggaggtggaggtggcagtggaggaattgcagaagctggaagtggtcatatgaactacattcaagtaacacctcaggaaaaagaagctatagaaaggttaaaggcattaggatttcctgaaggacttgtgatacaagcgtattttgcttgtgagaagaatgagaatttggctgccaattttcttctacagcagaactttgatgaagat

SEQ ID NO: 16 - DNA, 624 bp, Homo sapiens
atggacccgttcctggtgctgctgcactcggtgtcgtccagcctgtcgagcagcgagctgaccgagctcaagttcctatgcctcgggcgcgtgggcaagcgcaagctggagcgcgtgcagagcggcctagacctcttctccatgctgctggagcagaacgacctggagcccgggcacaccgagctcctgcgcgagctgctcgcctccctgcggcgccacgacctgctgcggcgcgtcgacgacttcgaggcgggggcggcggccggggccgcgcctggggaagaagacctgtgtgcagcatttaacgtcatatgtgataatgtggggaaagattggagaaggctggctcgtcagctcaaagtctcagacaccaagatcgacagcatcgaggacagatacccccgcaacctgacagagcgtgtgcgggagtcactgagaatctggaagaacacagagaaggagaacgcaacagtggcccacctggtgggggctctcaggtcctgccagatgaacctggtggctgacctggtacaagaggttcagcaggcccgtgacctccagaacaggagtggggccatgtccccgatgtcatggaactcagacgcatctacctccgaagcgtcc

SEQ ID NO: 17 - DNA, 678 bp, Homo sapiens
atgtcctccccccgtgacttccgtgctgagcccgtgaacgactacgagggcaacgactccgaggctgaggacctgaacttccgtgaaaccctgccctccagctcccaagagaacaccccccgttccaaggtgttcgagaacaaggtcaactccgagaaggtcaagctgtccctgcgcaacttcccccacaacgattacgaggacgtgttcgaggaaccctccgagtccggttccgacccctccatgtggaccgctcgtggtcccttccgtcgtgaccgttggtcctccgaggacgaggaagctgctggaccctcccaggctctgtcccccctgctgtccgacacccgcaagatcgtgtccgagggcgagctggaccagctggctcagatccgtcccctgatcttcaacttccacgagcagaccgctatcaaggactgcctgaagatcctcgaggaaaagaccgctgcttacgacatcatgcaagagttcatggctctcgagctgaagaacctgcccggcgagttcaactccggcaaccagccctccaaccgcgagaagaaccgttaccgtgacatcctgcctttccagcaccacggttactccggtcccaacgagcgtaccaccttctggcacggttccaacgagggtgctgtgtccctgctgctgcgctactgcgct

SEQ ID NO: 18 - DNA, 852 bp, Homo sapiens
atggacgccatcaagaagaagatgcagatgctgaagctcgacaaggagaacgccttggatcgagctgagcaggcggaggccgacaagaaggcggcggaagacaggagcaagcagctggaagatgagctggtgtcactgcaaaagaaactcaagggcaccgaagatgaactggacaaatattctgaggctctcaaagatgcccaggagaagctggagctggcagagaaaaaggccaccgatgctgaagccgacgtagcttctctgaacagacgcatccagctggttgaggaagagttggatcgtgcccaggagcgtctggcaacagctttgcagaagctggaggaagctgagaaggcagcagatgagagtgagagaggcatgaaagtcattgagagtcgagcccaaaaagatgaagaaaaaatggaaattcaggagatccaactgaaagaggcaaagcacattgctgaagatgccgaccgcaaatatgaagaggtggcccgtaagctggtcatcattgagagcgacctggaacgtgcagaggagcgggctgagctctcagaaggccaagtccgacagctggaagaacaattaagaataatggatcagaccttgaaagcattaatggctgcagaggataagtactcgcagaaggaagacagatatgaggaagagatcaaggtcctttccgacaagctgaaggaggctgagactcgggctgagtttgcggagaggtcagtaactaaattggagaaaagcattgatgacttagaagacgagctgtacgctcagaaactgaagtacaaagccatcagcgaggagctggaccacgctctcaacgatatgacttccatg

SEQ ID NO: 19 - DNA, 540 bp, Homo sapiens
atgcaggctgagggtcgtggcaccggtggttccactggcgacgctgacggtcccggtggtcctggtatccccgacggtcctggtggcaacgctggtggtccaggcgaggctggtgctaccggtggtcgtggtcctcgtggtgctggtgctgctcgtgcttccggtccaggtggtggtgctccccgtggtcctcacggtggtgctgcttccggcctgaacggttgctgccgttgcggtgctcgcggtcccgagtcccgtctgctcgagttctacctggctatgcccttcgctacccctatggaagctgagctggctcgtcgttccctggctcaggacgctcctcctctgcccgtgcccggtgtcctgctgaaggagttcactgtctccggcaacatcctgaccatccgtctgaccgctgctgaccaccgtcagctccagctgtccatctcctcatgcctgcagcagctgtccctgctgatgtggatcacccagtgtttcttgcccgtgttcctggctcagcccccctccggtcaacgtcgt

SEQ ID NO: 20 - protein, 81 aa, Homo sapiens
MESPKKKNQQLKVGILHLGSRQKKIRIQLRSQCATWKVICKSCISQTPGINLDLGSGVKVKIIPKEEHCKMPEAGEEQPQV

SEQ ID NO: 21 - protein, 400 aa, Homo sapiens
MGTPASGRKRTPVKDRFSAEDEALSNIAREAEARLAAKRAARAEARDIRMRELERQQKELDEKSDKQYAENYTRPSSRNSASATTPLSGNSSRRGSGDTSSLIDPDTSLSELRESLSEVEEKYKKAMVSNAQLDNEKNNLIYQVDTLKDVIEEQEEQMAEFYRENEEKSKELERQKHMCSVLQHKMEELKEGLRQRDELIEKHGLVIIPDGTPNGDVSHEPVAGAITVVSQEAAQVLESAGEGPLDVRLRKLAGEKEELLSQIRKLKLQLEEERQKCSRNDGTVGDLAGLQNGSDLQFIEMQRDANRQISEYKFKLSKAEQDITTLEQSISRLEGQVLRYKTAAENAEKVEDELKAEKRKLQRELRTALDKIEEMEMTNSHLAKRLEKMKANRTALLAQQ

SEQ ID NO: 22 - protein, 116 aa, Homo sapiens
MSWRGRSTYRPRPRRYVEPPEMIGPMRPEQFSDEVEPATPEEGEPATQRQDPAAAQEGEDEGASAGQGPKPEAHSQEQGHPQTGCECEDGPDGQEMDPPNPEEVKTPEEGEKQSQC

SEQ ID NO: 23 - protein, 631 aa, Homo sapiens
MSHWAPEWKRAEANPRDLGASWDVRGSRGSGWSGPFGHQGPRAAGSREPPLCFKIKNNMVGVVIGYSGSKIKDLQHSTNTKIQIINGESEAKVRIFGNREMKAKAKAAIETLIRKQESYNSESSVDNAASQTPIGRNLGRNDIVGEAEPLSNWDRIRAAVVECEKRKWADLPPVKKNFYIESKATSCMSEMQVINWRKENFNITCDDLKSGEKRLIPKPTCRFKDAFQQYPDLLKSIIRVGIVKPTPIQSQAWPIILQGIDLIVVAQTGTGKTLSYLMPGFIHLDSQPISREQRNGPGMLVLTPTRELALHVEAECSKYSYKGLKSICIYGGRNRNGQIEDISKGVDIIIATPGRLNDLQMNNSVNLRSITYLVIDEADKMLDMEFEPQIRKILLDVRPDRQTVMTSATWPDTVRQLALSYLKDPMIVYVGNLNLVAVNTVKQNIIVTTEKEKRALTQEFVENMSPNDKVIMFVSQKHIADDLSSDFNIQGISAESLHGNSEQSDQERAVEDFKSGNIKILITTDIVSRGLDLNDVTHVYNYDFPRNIDVYVHRVGYIGRTGKTGTSVTLITQRDSKMAGELIKILDRANQSVPEDLVVMAEQYKLNQQKRHRETRSRKPGQRRKEFYFLS

SEQ ID NO: 24 - protein, 648 aa, Homo sapiens
MSHHGGAPKASTWVVASRRSSTVSRAPERRPAEELNRTGPEGYSVGRGGRWRGTSRPPEAVAAGHEELPLCFALKSHFVGAVIGRGGSKIKNIQSTTNTTIQIIQEQPESLVKIFGSKAMQTKAKAVIDNFVKKLEENYNSECGIDTAFQPSVGKDGSTDNNVVAGDRPLIDWDQIREEGLKWQKTKWADLPPIKKNFYKESTATSAMSKVEADSWRKENFNITWDDLKDGEKRPIPNPTCTFDDAFQCYPEVMENIKKAGFQKPTPIQSQAWPIVLQGIDLIGVAQTGTGKTLCYLMPGFIHLVLQPSLKGQRNRPGMLVLTPTRELALQVEGECCKYSYKGLRSVCVYGGGNRDEQIEELKKGVDIIIATPGRLNDLQMSNFVNLKNITYLVLDEADKMLDMGFEPQIMKILLDVRPDRQTVMTSATWPHSVHRLAQSYLKEPMIVYVGTLDLVAVSSVKQNIIVTTEEEKWSHMQTFLQSMSSTDKVIVFVSRKAVADHLSSDLILGNISVESLHGDREQRDREKALENFKTGKVRILIATDLASRGLDVHDVTHVYNFDFPRNIEEYVHRIGRTGRAGRTGVSITTLTRNDWRVASELINILERANQSIPEELVSMAERFKAHQQKREMERKMERPQGRPKKFH

SEQ ID NO: 25 - protein, 139 aa, Homo sapiens
MSWRGRSTYYWPRPRRYVQPPEMIGPMRPEQFSDEVEPATPEEGEPATQRQDPAAAQEGEDEGASAGQGPKPEADSQEQGHPQTGCECEDGPDGQEMDPPNPEEVKTPEEEMRSHYVAQTGILWLLMNNCFLNLSPRKP

SEQ ID NO: 26 - protein, 369 aa, Homo sapiens
MPRAPKRQRCMPEEDLQSQSETQGLEGAQAPLAVEEDASSSTSTSSSFPSSFPSSSSSSSSSCYPLIPSTPEEVSADDETPNPPQSAQIACSSPSVVASLPLDQSDEGSSSQKEESPSTLQVLPDSESLPRSEIDEKVTDLVQFLLFKYQMKEPITKAEILESVIRNYEDHFPLLFSEASECMLLVFGIDVKEVDPTGHSFVLVTSLGLTYDGMLSDVQSMPKTGILILILSIVFIEGYCTPEEVIWEALNMMGLYDGMEHLIYGEPRKLLTQDWVQENYLEYRQVPGSDPARYEFLWGPRAHAEIRKMSLLKFLAKVNGSDPRSFPLWYEEALKDEEERAQDRIATTDDTTAMASASSSATGSFSYPE

SEQ ID NO: 27 - protein, 126 aa, Homo sapiens
MSVMDLANTCSSFQSDLDFCSDCGSVLPLPGAQDTVTCIRCGFNINVRDFEGKVVKTSVVFHQLGTAMPMSVEEGPECQGPVVDRRCPRCGHEGMAYHTRQMRSADEGQTVFYTCTNCKFQEKEDS

SEQ ID NO: 28 - protein, 448 aa, Homo sapiens
MLWLALGPFPAMENQVLVIRIKIPNSGAVDWTVHSGPQLLFRDVLDVIGQVLPEATTTAFEYEDEDGDRITVRSDEEMKAMLSYYYSTVMEQQVNGQLIEPLQIFPRACKPPGERNIHGLKVNTRAGPSQHSSPAVSDSLPSNSLKKSSAELKKILANGQMNEQDIRYRDTLGHGNGGTVYKAYHVPSGKILAVKVILLDITLELQKQIMSELEILYKCDSSYIIGFYGAFFVENRISICTEFMDGGSLDVYRKMPEHVLGRIAVAVVKGLTYLWSLKILHRDVKPSNMLVNTRGQVKLCDFGVSTQLVNSIAKTYVGTNAYMAPERISGEQYGIHSDVWSLGISFMELALGRFPYPQIQKNQGSLMPLQLLQCIVDEDSPVLPVGEFSEPFVHFITQCMRKQPKERPAPEELMGHPFIVQFNDGNAAVVSMWVCRALEERRSQQGPP

SEQ ID NO: 29 - protein, 317 aa, Homo sapiens
MSSEQKSQHCKPEEGVEAQEEALGLVGAQAPTTEEQEAAVSSSSPLVPGTLEEVPAAESAGPPQSPQGASALPTTISFTCWRQPNEGSSSQEEEGPSTSPDAESLFREALSNKVDELAHFLLRKYRAKELVTKAEMLERVIKNYKRCFPVIFGKASESLKMIFGIDVKEVDPASNTYTLVTCLGLSYDGLLGNNQIFPKTGLLIIVLGTIAMEGDSASEEEIWEELGVMGVYDGREHTVYGEPRKLLTQDWVQENYLEYRQVPGSNPARYEFLWGPRALAETSYVKVLEHVVRVNARVRIAYPSLREAALLEEEEGV

SEQ ID NO: 30 - protein, 712 aa, Homo sapiens
MSQWYELQQLDSKFLEQVHQLYDDSFPMEIRQYLAQWLEKQDWEHAANDVSFATIRFHDLLSQLDDQYSRFSLENNFLLQHNIRKSKRNLQDNFQEDPIQMSMIIYSCLKEERKILENAQRFNQAQSGNIQSTVMLDKQKELDSKVRNVKDKVMCIEHEIKSLEDLQDEYDFKCKTLQNREHETNGVAKSDQKQEQLLLKKMYLMLDNKRKEVVHKIIELLNVTELTQNALINDELVEWKRRQQSACIGGPPNACLDQLQNWFTIVAESLQQVRQQLKKLEELEQKYTYEHDPITKNKQVLWDRTFSLFQQLIQSSFVVERQPCMPTHPQRPLVLKTGVQFTVKLRLLVKLQELNYNLKVKVLFDKDVNERNTVKGFRKFNILGTHTKVMNMEESTNGSLAAEFRHLQLKEQKNAGTRTNEGPLIVTEELHSLSFETQLCQPGLVIDLETTSLPVVVISNVSQLPSGWASILWYNMLVAEPRNLSFFLTPPCARWAQLSEVLSWQFSSVTKRGLNVDQLNMLGEKLLGPNASPDGLIPWTRFCKENINDKNFPFWLWIESILELIKKHLLPLWNDGCIMGFISKERERALLKDQQPGTFLLRFSESSREGAITFTWVERSQNGGEPDFHAVEPYTKKELSAVTFPDIIRNYKVMAAENIPENPLKYLYPNIDKDHAFGKYYSRPKEAPEPMELDGPKGTGYIKTELISVSEV

SEQ ID NO: 31 - protein, 288 aa, Homo sapiens
MSATGDRHPTQGDQEAPVSQEGAQAEAAGAGNQEGGDSGPDSSDVVPAAEVVGVAGPVEGLGEEEGEQAAGLAAVPRGGSAEEDSDIGPATEEEEEEEGNEAANFDLAVVARRYPASGIHFVLLDMVHSLLHRLSHNDHILIENRQLSRLMVGPHAAARNLWGNLPPLLLPQRLGAGAAARAGEGLGLIQEAASVPEPAVPADLAEMAREPAEEAAEEKLSEEATEEPDAEEPATEEPTAQEATAPEEVTKSQPEKWDEEAQDAAGEEEKEQEKEKDAENKVKNSKGT

SEQ ID NO: 32 - protein, 579 aa, Homo sapiens
MNKLYIGNLSENAAPSDLESIFKDAKIPVSGPFLVKTGYAFVDCPDESWALKAIEALSGKIELHGKPIEVEHSVPKRQRIRKLQIRNIPPHLQWEVLDSLLVQYGVVESCEQVNTDSETAVVNVTYSSKDQARQALDKLNGFQLENFTLKVAYIPDEMAAQQNPLQQPRGRRGLGQRGSSRQGSPGSVSKQKPCDLPLRLLVPTQFVGAIIGKEGATIRNITKQTQSKIDVHRKENAGAAEKSITILSTPEGTSAACKSILEIMHKEAQDIKFTEEIPLKILAHNNFVGRLIGKEGRNLKKIEQDTDTKITISPLQELTLYNPERTITVKGNVETCAKAEEEIMKKIRESYENDIASMNLQAHLIPGLNLNALGLFPPTSGMPPPTSGPPSAMTPPYPQFEQSETETVHLFIPALSVGAIIGKQGQHIKQLSRFAGASIKIAPAEAPDAKVRMVIITGPPEAQFKAQGRIYGKIKEENFVSPKEEVKLEAHIRVPSFAAGRVIGKGGKTVNELQNLSSAEVVVPRDQTPDENDQVVVKITGHFYACQVAQRKIQEILTQVKQHQQQKALQSGPPQSRRK

SEQ ID NO: 33 - protein, 210 aa, Homo sapiens
MQAEGQGTGGSTGDADGPGGPGIPDGPGGNAGGPGEAGATGGRGPRGAGAARASGPRGGAPRGPHGGAASAQDGRCPCGARRPDSRLLQLHITMPFSSPMEAELVRRILSRDAAPLPRPGAVLKDFTVSGNLLFMSVRDQDREGAGRMRVVGWGLGSASPEGQKARDLRTPKHKVSEQRPGTPGPPPPEGAQGDGCRGVAFNVMFSAPHI

SEQ ID NO: 34 - protein, 409 aa, Homo sapiens
MQVTLKTLQQQTFKIDIDPEETVKALKEKIESEKGKDAFPVAGQKLIYAGKILNDDTALKEYKIDEKNFVVVMVTKPKAVSTPAPATTQQSAPASTTAVTSSTTTTVAQAPTPVPALAPTSTPASITPASATASSEPAPASAAKQEKPAEKPAETPVATSPTATDSTSGDSSRSNLFEDATSALVTGQSYENMVTEIMSMGYEREQVIAALRASFNNPDRAVEYLLMGIPGDRESQAVVDPPQAASTGAPQSSAVAAAAATTTATTTTTSSGGHPLEFLRNQPQFQQMRQIIQQNPSLLPALLQQIGRENPQLLQQISQHQEHFIQMLNEPVQEAGGQGGGGGGGSGGIAEAGSGHMNYIQVTPQEKEAIERLKALGFPEGLVIQAYFACEKNENLAANFLLQQNFDED

SEQ ID NO: 35 - protein, 208 aa, Homo sapiens
MDPFLVLLHSVSSSLSSSELTELKFLCLGRVGKRKLERVQSGLDLFSMLLEQNDLEPGHTELLRELLASLRRHDLLRRVDDFEAGAAAGAAPGEEDLCAAFNVICDNVGKDWRRLARQLKVSDTKIDSIEDRYPRNLTERVRESLRIWKNTEKENATVAHLVGALRSCQMNLVADLVQEVQQARDLQNRSGAMSPMSWNSDASTSEAS

SEQ ID NO: 36 - protein, 420 aa, Homo sapiens
MSSPRDFRAEPVNDYEGNDSEAEDLNFRETLPSSSQENTPRSKVFENKVNSEKVKLSLRNFPHNDYEDVFEEPSESGSDPSMWTARGPFRRDRWSSEDEEAAGPSQALSPLLSDTRKIVSEGELDQLAQIRPLIFNFHEQTAIKDCLKILEEKTAAYDIMQEFMALELKNLPGEFNSGNQPSNREKNRYRDILPYDSTRVPLGKSKDYINASYIRIVNCGEEYFYIATQGPLLSTIDDFWQMVLENNSNVIAMITREIEGGIIKCYHYWPISLKKPLELKHFRVFLENYQILQYFIIRMFQVVEKSTGTSHSVKQLQFTKWPDHGTPASADSFIKYIRYARKSHLTGPMVVHCSAGIGRTGVFLCVDVVFCAIVKNCSFNIMDIVAQMREQRSGMVQTKEQYHFCYDIVLEVLRKLLTLD

SEQ ID NO: 37 - protein, 284 aa, Homo sapiens
MDAIKKKMQMLKLDKENALDRAEQAEADKKAAEDRSKQLEDELVSLQKKLKGTEDELDKYSEALKDAQEKLELAEKKATDAEADVASLNRRIQLVEEELDRAQERLATALQKLEEAEKAADESERGMKVIESRAQKDEEKMEIQEIQLKEAKHIAEDADRKYEEVARKLVIIESDLERAEERAELSEGKCAELEEELKTVTNNLKSLEAQAEKYSQKEDRYEEEIKVLSDKLKEAETRAEFAERSVTKLEKSIDDLEDELYAQKLKYKAISEELDHALNDMTSI

SEQ ID NO: 38 - protein, 180 aa, Homo sapiens
MQAEGRGTGGSTGDADGPGGPGIPDGPGGNAGGPGEAGATGGRGPRGAGAARASGPGGGAPRGPHGGAASGLNGCCRCGARGPESRLLEFYLAMPFATPMEAELARRSLAQDAPPLPVPGVLLKEFTVSGNILTIRLTAADHRQLQLSISSCLQQLSLLMWITQCFLPVFLAQPPSGQRR